European Patent Application EP 4 640 700 A1, published October 29, 2025. Title: “KAPPA/LAMBDA" FAB-FAB SERIES-CONNECTION MULTI-SPECIFIC BINDING PROTEIN, PREPARATION THEREOF, AND USE THEREOF. Applicant: HARBOUR BIOMED(SHANGHAI) CO.,LTD. Application US, filed December 18, 2023. The sequence listing filed with the application follows.

SEQUENCE LISTING (196 sequences)

SEQ ID NO: 1 - protein, 25 aa, synthetic construct
EVQLVQSGAEVKKPGASVKVSCKAS

SEQ ID NO: 2 - protein, 25 aa, synthetic construct
EVQLVESGGGLVQPKGSLKLSCAAS

SEQ ID NO: 3 - protein, 25 aa, synthetic construct [sequence omitted]

SEQ ID NO: 4 - protein, 25 aa, synthetic construct
EVQLQQSGAELMKPGASVKISCKAS

SEQ ID NO: 5 - protein, 25 aa, synthetic construct
QVQLVESGGGLVKPGESLRLSCAAS

SEQ ID NO: 6 - protein, 25 aa, synthetic construct
EVQLVESGGGLVQPGRSLRLSCTAS

SEQ ID NO: 7 - protein, 25 aa, synthetic construct
EVQLVQSGAEVKKPGESLRISCKGS

SEQ ID NO: 8 - protein, 25 aa, synthetic construct
EVQLVESGGGLVQPGGSLKLSCAAS

SEQ ID NO: 9 - protein, 25 aa, synthetic construct [sequence omitted]

SEQ ID NO: 10 - protein, 25 aa, synthetic construct
EVQLLESGGGLVQPGGSLRLSCAAS

SEQ ID NO: 11 - protein, 25 aa, synthetic construct
QVQLVQSGAEVKKPGESLKVSCKAS

SEQ ID NO: 12 - protein, 7 aa, synthetic construct
GYTFTSY

SEQ ID NO: 13 - protein, 7 aa, synthetic construct
GFTFNTY

SEQ ID NO: 14 - protein, 7 aa, synthetic construct
GGTFSNY

SEQ ID NO: 15 - protein, 7 aa, synthetic construct
GYTFSDY

SEQ ID NO: 16 - protein, 7 aa, synthetic construct
GFTFSDY

SEQ ID NO: 17 - protein, 7 aa, synthetic construct
GSDINDY

SEQ ID NO: 18 - protein, 7 aa, synthetic construct
GYSFSTY

SEQ ID NO: 19 - protein, 7 aa, synthetic construct
GGSFSGY

SEQ ID NO: 20 - protein, 7 aa, synthetic construct
GFTFRSF

SEQ ID NO: 21 - protein, 7 aa, synthetic construct
GFTFSTY

SEQ ID NO: 22 - protein, 19 aa, synthetic construct
WIGWVRQAPGQGLEWIGDI

SEQ ID NO: 23 - protein, 19 aa, synthetic construct
AMNWVRQAPGKGLEWVARI

SEQ ID NO: 24 - protein, 19 aa, synthetic construct
WMHWVRQAPGQGLEWMGAT

SEQ ID NO: 25 - protein, 19 aa, synthetic construct
WIEWVKQRPGHGLEWIGEI

SEQ ID NO: 26 - protein, 19 aa, synthetic construct
YMYWVRQAPGKGLEWVAII

SEQ ID NO: 27 - protein, 19 aa, synthetic construct
PITWVRQAPGQGLEWIGFI

SEQ ID NO: 28 - protein, 19 aa, synthetic construct
WISWVRQMPGKGLEWMGKI

SEQ ID NO: 29 - protein, 19 aa, synthetic construct
AMNWVRQASGKGLEWVGRI

SEQ ID NO: 30 - protein, 19 aa, synthetic construct
YWSWIRQSPEKGLEWIGEI

SEQ ID NO: 31 - protein, 19 aa, synthetic construct
GMSWVRQAPGKGPEWVSSI

SEQ ID NO: 32 - protein, 19 aa, synthetic construct
YMHWVRQAPGQGLEWMGAI

SEQ ID NO: 33 - protein, 19 aa, synthetic construct
YMHWVRQAPGQGLEWMGII

SEQ ID NO: 34 - protein, 19 aa, synthetic construct
AMNWVRQAPGKGLEWVSRI

SEQ ID NO: 35 - protein, 6 aa, synthetic construct
YPGGGY

SEQ ID NO: 36 - protein, 8 aa, synthetic construct
RSKYNNYA

SEQ ID NO: 37 - protein, 6 aa, synthetic construct
YRGHSD

SEQ ID NO: 38 - protein, 6 aa, synthetic construct
LPGSGS

SEQ ID NO: 39 - protein, 6 aa, synthetic construct
SDGGYY

SEQ ID NO: 40 - protein, 5 aa, synthetic construct
NSGGS

SEQ ID NO: 41 - protein, 6 aa, synthetic construct
YPGDSY

SEQ ID NO: 42 - protein, 5 aa, synthetic construct
NHGGY

SEQ ID NO: 43 - protein, 6 aa, synthetic construct
SGSGSD

SEQ ID NO: 44 - protein, 6 aa, synthetic construct
EPMYGS

SEQ ID NO: 45 - protein, 6 aa, synthetic construct
NPSGGS

SEQ ID NO: 46 - protein, 41 aa, synthetic construct
TNYNEKFKGRVTITRDTSTSTAYLELSSLRSEDTAVYYCAR

SEQ ID NO: 47 - protein, 41 aa, synthetic construct
TYYADSVKDRFTISRDDSQSILYLQMNNLKTEDTAMYYCVR

SEQ ID NO: 48 - protein, 41 aa, synthetic construct
TYYNQKFKGRVTITADKSTSTAYMELSSLRSEDTAVYYCAR

SEQ ID NO: 49 - protein, 41 aa, synthetic construct
TNYHERFKGKATFTADTSSSTAYMQLNSLTSEDSGVYYCLH

SEQ ID NO: 50 - protein, 41 aa, synthetic construct
TYYSDIIKGRFTISRDNAKNSLYLQMNSLKAEDTAVYYCAR

SEQ ID NO: 51 - protein, 41 aa, synthetic construct
TWYASWVKGRFTISRDDSKSIAYLQMNSLKTEDTAVYYCAR

SEQ ID NO: 52 - protein, 41 aa, synthetic construct
TNYSPSFQGQVTISADKSISTAYLQWSSLKASDTAMYYCAR

SEQ ID NO: 53 - protein, 41 aa, synthetic construct
TYYADSVKDRFTISRDDSKSTLYLQMNSLKTEDTAVYYCVR

SEQ ID NO: 54 - protein, 41 aa, synthetic construct
VTYNPSLESRVTISVDTSKNQFSLKLSSVTAADTAVYYCAR

SEQ ID NO: 55 - protein, 41 aa, synthetic construct
TLYADSVKGRFTISRDNSKNTLYLQMNSLRPEDTAVYYCTI

SEQ ID NO: 56 - protein, 41 aa, synthetic construct
TSYAQKFQGRVTMTRDTSTSTVYMELSSLRSEDTAVYYCAR

SEQ ID NO: 57 - protein, 41 aa, synthetic construct
TYYADSVKDRFTISRDDSKSTLYLQMNSLRAEDTAVYYCVR

SEQ ID NO: 58 - protein, 12 aa, synthetic construct
LAGSSYRGAMDS

SEQ ID NO: 59 - protein, 14 aa, synthetic construct
HGNFGNSYVSWFAY

SEQ ID NO: 60 - protein, 12 aa, synthetic construct
GAIYDGYDVLDN

SEQ ID NO: 61 - protein, 7 aa, synthetic construct
GNYDFDG

SEQ ID NO: 62 - protein, 12 aa, synthetic construct
GFPLLRHGAMDY

SEQ ID NO: 63 - protein, 11 aa, synthetic construct
GYSTYYRDFNI

SEQ ID NO: 64 - protein, 7 aa, synthetic construct
GYGIFDY

SEQ ID NO: 65 - protein, 13 aa, synthetic construct
DYGPGNYDWYFDL

SEQ ID NO: 66 - protein, 6 aa, synthetic construct
GGSLSR

SEQ ID NO: 67 - protein, 11 aa, synthetic construct
GSAYYYDFADY

SEQ ID NO: 68 - protein, 11 aa, synthetic construct
WGQGTLVTVSS

SEQ ID NO: 69 - protein, 11 aa, synthetic construct
WGQGTLVTVSA

SEQ ID NO: 70 - protein, 11 aa, synthetic construct
WGQGTTLTVSS

SEQ ID NO: 71 - protein, 11 aa, synthetic construct
WGRGTLVTVSS

SEQ ID NO: 72 - protein, 11 aa, synthetic construct
SSQGTLVTVSS

SEQ ID NO: 73 - protein, 23 aa, synthetic construct
DIQMTQSPSSLSASVGDRVTITC

SEQ ID NO: 74 - protein, 22 aa, synthetic construct
QAVVTQESALTTSPGETVTLTC

SEQ ID NO: 75 - protein, 23 aa, synthetic construct
DIVLTQSPAIMSASPGEKVTMTC

SEQ ID NO: 76 - protein, 23 aa, synthetic construct
DIQMTQSPSSLSASVGDRVTINC

SEQ ID NO: 77 - protein, 22 aa, synthetic construct
SYELTQPPSVSVSPGQTASITC

SEQ ID NO: 78 - protein, 22 aa, synthetic construct
QAVVTQEPSLTVSPGGTVTLTC

SEQ ID NO: 79 - protein, 23 aa, synthetic construct
EIVLTQSPATLSLSPGERATLSC

SEQ ID NO: 80 - protein, 22 aa, synthetic construct
SYVLTQPSSVSVAPGQTATISC

SEQ ID NO: 81 - protein, 11 aa, synthetic construct
KASQGFNKYVA

SEQ ID NO: 82 - protein, 14 aa, synthetic construct
RSSTGAVTTSNYAN

SEQ ID NO: 83 - protein, 11 aa, synthetic construct
SASQDISNYLN

SEQ ID NO: 84 - protein, 10 aa, synthetic construct
SASSSVNYMY

SEQ ID NO: 85 - protein, 11 aa, synthetic construct
KASQNVDTNVA

SEQ ID NO: 86 - protein, 11 aa, synthetic construct
QASQSIDSNLA

SEQ ID NO: 87 - protein, 11 aa, synthetic construct
SGDNIGDQYAH

SEQ ID NO: 88 - protein, 11 aa, synthetic construct
RASQSVSSYLA

SEQ ID NO: 89 - protein, 11 aa, synthetic construct
GGHNIGSKNVH

SEQ ID NO: 90 - protein, 15 aa, synthetic construct
WYQQKPGKAPKLLIY

SEQ ID NO: 91 - protein, 15 aa, synthetic construct
WVQEKPDHLFTGLIG

SEQ ID NO: 92 - protein, 15 aa, synthetic construct
WYQQKSGTSPKRWIY

SEQ ID NO: 93 - protein, 15 aa, synthetic construct
WYQQKPGQAPKSLIY

SEQ ID NO: 94 - protein, 15 aa, synthetic construct
WFQQKPGQPPKLLIY

SEQ ID NO: 95 - protein, 15 aa, synthetic construct
WYQQKPGQSPVLVIY

SEQ ID NO: 96 - protein, 15 aa, synthetic construct
WVQQKPGQAPRGLIG

SEQ ID NO: 97 - protein, 15 aa, synthetic construct
WYQQKPGQAPRLLIY

SEQ ID NO: 98 - protein, 15 aa, synthetic construct
WYQQRPGQSPVLVIY

SEQ ID NO: 99 - protein, 7 aa, synthetic construct
YTSTLQP

SEQ ID NO: 100 - protein, 7 aa, synthetic construct
GTNKRAP

SEQ ID NO: 101 - protein, 7 aa, synthetic construct
YTSNLHS

SEQ ID NO: 102 - protein, 7 aa, synthetic construct
DTSKLAS

SEQ ID NO: 103 - protein, 7 aa, synthetic construct
SASYRYS

SEQ ID NO: 104 - protein, 7 aa, synthetic construct
RASNLAS

SEQ ID NO: 105 - protein, 7 aa, synthetic construct
QDKNRPS

SEQ ID NO: 106 - protein, 7 aa, synthetic construct
DASNRAT

SEQ ID NO: 107 - protein, 7 aa, synthetic construct
QDNKRPS

SEQ ID NO: 108 - protein, 32 aa, synthetic construct
GVPSRFSGSGSGRDYTLTISSLQPEDFATYYC

SEQ ID NO: 109 - protein, 32 aa, synthetic construct
GVPARFSGSLIGDKAALTITGAQTEDEAIYFC

SEQ ID NO: 110 - protein, 32 aa, synthetic construct
GVPSRFSGSGSGTDFTLTISSLQPEDFATYYC

SEQ ID NO: 111 - protein, 32 aa, synthetic construct
GVPVRFSGSGSGTSYSLTISSMETEDAAEYYC

SEQ ID NO: 112 - protein, 32 aa, synthetic construct
DVPSRFSGSASGTDFTLTISSVQSEDFATYYC

SEQ ID NO: 113 - protein, 32 aa, synthetic construct
GVPDRFSGSGSGTDFTLTISSLEAEDVATYYC

SEQ ID NO: 114 - protein, 32 aa, synthetic construct
GIPERFSGSNSGNTATLTISGTQAMDEADYYC

SEQ ID NO: 115 - protein, 32 aa, synthetic construct
WTPARFSGSLLGDKAALTLLGAQPEDEAEYFC

SEQ ID NO: 116 - protein, 32 aa, synthetic construct
GIPARFSGSGSGTDFTLTISSLEPEDFAVYYC

SEQ ID NO: 117 - protein, 9 aa, synthetic construct
LQYGDLLYA

SEQ ID NO: 118 - protein, 9 aa, synthetic construct
ALWYSNLWV

SEQ ID NO: 119 - protein, 9 aa, synthetic construct
QQYRKLPWT

SEQ ID NO: 120 - protein, 8 aa, synthetic construct
QQWGRNPT

SEQ ID NO: 121 - protein, 9 aa, synthetic construct
QQYDSYPYT

SEQ ID NO: 122 - protein, 12 aa, synthetic construct
LGGVGAVSYRTS

SEQ ID NO: 123 - protein, 11 aa, synthetic construct
ATYTGFGSLAV

SEQ ID NO: 124 - protein, 11 aa, synthetic construct
QQRSNWPPALT

SEQ ID NO: 125 - protein, 9 aa, synthetic construct
QVWDNYSVL

SEQ ID NO: 126 - protein, 10 aa, synthetic construct
FGQGTKVEIK

SEQ ID NO: 127 - protein, 10 aa, synthetic construct
FGGGTKLTVL

SEQ ID NO: 128 - protein, 10 aa, synthetic construct
FGQGTKLEIK

SEQ ID NO: 129 - protein, 10 aa, synthetic construct
FGGGTKLEIK

SEQ ID NO: 130 - protein, 10 aa, synthetic construct
FGGGTKVEIK

SEQ ID NO: 131 - protein, 121 aa, synthetic construct
EVQLVQSGAEVKKPGASVKVSCKASGYTFTSYWIGWVRQAPGQGLEWIGDIYPGGGYTNYNEKFKGRVTITRDTSTSTAYLELSSLRSEDTAVYYCARLAGSSYRGAMDSWGQGTLVTVSS

SEQ ID NO: 132 - protein, 125 aa, synthetic construct
EVQLVESGGGLVQPKGSLKLSCAASGFTFNTYAMNWVRQAPGKGLEWVARIRSKYNNYATYYADSVKDRFTISRDDSQSILYLQMNNLKTEDTAMYYCVRHGNFGNSYVSWFAYWGQGTLVTVSA

SEQ ID NO: 133 - protein, 121 aa, synthetic construct
QVQLVQSGAEVKKPGSSVKVSCKASGGTFSNYWMHWVRQAPGQGLEWMGATYRGHSDTYYNQKFKGRVTITADKSTSTAYMELSSLRSEDTAVYYCARGAIYDGYDVLDNWGQGTLVTVSS

SEQ ID NO: 134 - protein, 116 aa, synthetic construct
EVQLQQSGAELMKPGASVKISCKASGYTFSDYWIEWVKQRPGHGLEWIGEILPGSGSTNYHERFKGKATFTADTSSSTAYMQLNSLTSEDSGVYYCLHGNYDFDGWGQGTTLTVSS

SEQ ID NO: 135 - protein, 121 aa, synthetic construct
QVQLVESGGGLVKPGESLRLSCAASGFTFSDYYMYWVRQAPGKGLEWVAIISDGGYYTYYSDIIKGRFTISRDNAKNSLYLQMNSLKAEDTAVYYCARGFPLLRHGAMDYWGQGTLVTVSS

SEQ ID NO: 136 - protein, 119 aa, synthetic construct
EVQLVESGGGLVQPGRSLRLSCTASGSDINDYPITWVRQAPGQGLEWIGFINSGGSTWYASWVKGRFTISRDDSKSIAYLQMNSLKTEDTAVYYCARGYSTYYRDFNIWGQGTLVTVSS

SEQ ID NO: 137 - protein, 116 aa, synthetic construct
EVQLVQSGAEVKKPGESLRISCKGSGYSFSTYWISWVRQMPGKGLEWMGKIYPGDSYTNYSPSFQGQVTISADKSISTAYLQWSSLKASDTAMYYCARGYGIFDYWGQGTLVTVSS

SEQ ID NO: 138 - protein, 125 aa, synthetic construct
EVQLVESGGGLVQPGGSLKLSCAASGFTFNTYAMNWVRQASGKGLEWVGRIRSKYNNYATYYADSVKDRFTISRDDSKSTLYLQMNSLKTEDTAVYYCVRHGNFGNSYVSWFAYWGQGTLVTVSS

SEQ ID NO: 139 - protein, 121 aa, synthetic construct [sequence omitted]

SEQ ID NO: 140 - protein, 115 aa, synthetic construct [sequence omitted]

SEQ ID NO: 141 - protein, 120 aa, synthetic construct
QVQLVQSGAEVKKPGESLKVSCKASGYTFTSYYMHWVRQAPGQGLEWMGAIEPMYGSTSYAQKFQGRVTMTRDTSTSTVYMELSSLRSEDTAVYYCARGSAYYYDFADYWGQGTLVTVSS

SEQ ID NO: 142 - protein, 120 aa, synthetic construct
QVQLVQSGAEVKKPGESLKVSCKASGYTFTSYYMHWVRQAPGQGLEWMGIINPSGGSTSYAQKFQGRVTMTRDTSTSTVYMELSSLRSEDTAVYYCARGSAYYYDFADYWGQGTLVTVSS

SEQ ID NO: 143 - protein, 125 aa, synthetic construct
EVQLLESGGGLVQPGGSLRLSCAASGFTFSTYAMNWVRQAPGKGLEWVSRIRSKYNNYATYYADSVKDRFTISRDDSKSTLYLQMNSLRAEDTAVYYCVRHGNFGNSYVSWFAYWGQGTLVTVSS

SEQ ID NO: 144 - protein, 107 aa, synthetic construct
DIQMTQSPSSLSASVGDRVTITCKASQGFNKYVAWYQQKPGKAPKLLIYYTSTLQPGVPSRFSGSGSGRDYTLTISSLQPEDFATYYCLQYGDLLYAFGQGTKVEIK

SEQ ID NO: 145 - protein, 109 aa, synthetic construct
QAVVTQESALTTSPGETVTLTCRSSTGAVTTSNYANWVQEKPDHLFTGLIGGTNKRAPGVPARFSGSLIGDKAALTITGAQTEDEAIYFCALWYSNLWVFGGGTKLTVL

SEQ ID NO: 146 - protein, 107 aa, synthetic construct
DIQMTQSPSSLSASVGDRVTITCSASQDISNYLNWYQQKPGKAPKLLIYYTSNLHSGVPSRFSGSGSGTDFTLTISSLQPEDFATYYCQQYRKLPWTFGQGTKLEIK

SEQ ID NO: 147 - protein, 105 aa, synthetic construct
DIVLTQSPAIMSASPGEKVTMTCSASSSVNYMYWYQQKSGTSPKRWIYDTSKLASGVPVRFSGSGSGTSYSLTISSMETEDAAEYYCQQWGRNPTFGGGTKLEIK

SEQ ID NO: 148 - protein, 107 aa, synthetic construct
DIQMTQSPSSLSASVGDRVTITCKASQNVDTNVAWYQQKPGQAPKSLIYSASYRYSDVPSRFSGSASGTDFTLTISSVQSEDFATYYCQQYDSYPYTFGGGTKLEIK

SEQ ID NO: 149 - protein, 110 aa, synthetic construct
DIQMTQSPSSLSASVGDRVTINCQASQSIDSNLAWFQQKPGQPPKLLIYRASNLASGVPDRFSGSGSGTDFTLTISSLEAEDVATYYCLGGVGAVSYRTSFGGGTKVEIK

SEQ ID NO: 150 - protein, 108 aa, synthetic construct
SYELTQPPSVSVSPGQTASITCSGDNIGDQYAHWYQQKPGQSPVLVIYQDKNRPSGIPERFSGSNSGNTATLTISGTQAMDEADYYCATYTGFGSLAVFGGGTKLTVL

SEQ ID NO: 151 - protein, 109 aa, synthetic construct
QAVVTQEPSLTVSPGGTVTLTCRSSTGAVTTSNYANWVQQKPGQAPRGLIGGTNKRAPWTPARFSGSLLGDKAALTLLGAQPEDEAEYFCALWYSNLWVFGGGTKLTVL

SEQ ID NO: 152 - protein, 109 aa, synthetic construct [sequence omitted]

SEQ ID NO: 153 - protein, 106 aa, synthetic construct
SYVLTQPSSVSVAPGQTATISCGGHNIGSKNVHWYQQRPGQSPVLVIYQDNKRPSGIPERFSGSNSGNTATLTISGTQAMDEADYYCQVWDNYSVLFGGGTKLTVL

SEQ ID NO: 154 - protein, 451 aa, synthetic construct
EVQLVQSGAEVKKPGASVKVSCKASGYTFTSYWIGWVRQAPGQGLEWIGDIYPGGGYTNYNEKFKGRVTITRDTSTSTAYLELSSLRSEDTAVYYCARLAGSSYRGAMDSWGQGTLVTVSSASTKGPSVFPLAPSSKSTSGGTAALGCLVKDYFPEPVTVSWNSGALTSGVHTFPAVLQSSGLYSLSSVVTVPSSSLGTQTYICNVNHKPSNTKVDKKVEPKSCDKTHTCPPCPAPELLGGPSVFLFPPKPKDTLMISRTPEVTCVVVDVSHEDPEVKFNWYVDGVEVHNAKTKPREEQYNSTYRVVSVLTVLHQDWLNGKEYKCKVSNKALPAPIEKTISKAKGQPREPQVYTLPPSREEMTKNQVSLTCLVKGFYPSDIAVEWESNGQPENNYKTTPPVLDSDGSFFLYSKLTVDKSRWQQGNVFSCSVMHEALHNHYTQKSLSLSPGK

SEQ ID NO: 155 - protein, 455 aa, synthetic construct
EVQLVESGGGLVQPKGSLKLSCAASGFTFNTYAMNWVRQAPGKGLEWVARIRSKYNNYATYYADSVKDRFTISRDDSQSILYLQMNNLKTEDTAMYYCVRHGNFGNSYVSWFAYWGQGTLVTVSAASTKGPSVFPLAPSSKSTSGGTAALGCLVKDYFPEPVTVSWNSGALTSGVHTFPAVLQSSGLYSLSSVVTVPSSSLGTQTYICNVNHKPSNTKVDKKVEPKSCDKTHTCPPCPAPEAAGGPSVFLFPPKPKDTLMISRTPEVTCVVVDVSHEDPEVKFNWYVDGVEVHNAKTKPREEQYNSTYRVVSVLTVLHQDWLNGKEYKCKVSNKALPAPIEKTISKAKGQPREPQVYTLPPSREEMTKNQVSLTCLVKGFYPSDIAVEWESNGQPENNYKTTPPVLDSDGSFFLYSKLTVDKSRWQQGNVFSCSVMHEALHNHYTQKSLSLSPGK

SEQ ID NO: 156 - protein, 451 aa, synthetic construct
QVQLVQSGAEVKKPGSSVKVSCKASGGTFSNYWMHWVRQAPGQGLEWMGATYRGHSDTYYNQKFKGRVTITADKSTSTAYMELSSLRSEDTAVYYCARGAIYDGYDVLDNWGQGTLVTVSSASTKGPSVFPLAPSSKSTSGGTAALGCLVKDYFPEPVTVSWNSGALTSGVHTFPAVLQSSGLYSLSSVVTVPSSSLGTQTYICNVNHKPSNTKVDKKVEPKSCDKTHTCPPCPAPELLGGPSVFLFPPKPKDTLMISRTPEVTCVVVDVSHEDPEVKFNWYVDGVEVHNAKTKPREEQYNSTYRVVSVLTVLHQDWLNGKEYKCKVSNKALPAPIEKTISKAKGQPREPQVYTLPPSREEMTKNQVSLTCLVKGFYPSDIAVEWESNGQPENNYKTTPPVLDSDGSFFLYSKLTVDKSRWQQGNVFSCSVMHEALHNHYTQKSLSLSPGK

SEQ ID NO: 157 - protein, 446 aa, synthetic construct
EVQLQQSGAELMKPGASVKISCKASGYTFSDYWIEWVKQRPGHGLEWIGEILPGSGSTNYHERFKGKATFTADTSSSTAYMQLNSLTSEDSGVYYCLHGNYDFDGWGQGTTLTVSSASTKGPSVFPLAPSSKSTSGGTAALGCLVKDYFPEPVTVSWNSGALTSGVHTFPAVLQSSGLYSLSSVVTVPSSSLGTQTYICNVNHKPSNTKVDKKVEPKSCDKTHTCPPCPAPELLGGPSVFLFPPKPKDTLMISRTPEVTCVVVDVSHEDPEVKFNWYVDGVEVHNAKTKPREEQYNSTYRVVSVLTVLHQDWLNGKEYKCKVSNKALPAPIEKTISKAKGQPREPQVYTLPPSREEMTKNQVSLTCLVKGFYPSDIAVEWESNGQPENNYKTTPPVLDSDGSFFLYSKLTVDKSRWQQGNVFSCSVMHEALHNHYTQKSLSLSPGK

SEQ ID NO: 158 - protein, 451 aa, synthetic construct
QVQLVESGGGLVKPGESLRLSCAASGFTFSDYYMYWVRQAPGKGLEWVAIISDGGYYTYYSDIIKGRFTISRDNAKNSLYLQMNSLKAEDTAVYYCARGFPLLRHGAMDYWGQGTLVTVSSASTKGPSVFPLAPSSKSTSGGTAALGCLVKDYFPEPVTVSWNSGALTSGVHTFPAVLQSSGLYSLSSVVTVPSSSLGTQTYICNVNHKPSNTKVDKKVEPKSCDKTHTCPPCPAPELLGGPSVFLFPPKPKDTLMISRTPEVTCVVVDVSHEDPEVKFNWYVDGVEVHNAKTKPREEQYNSTYRVVSVLTVLHQDWLNGKEYKCKVSNKALPAPIEKTISKAKGQPREPQVYTLPPSREEMTKNQVSLTCLVKGFYPSDIAVEWESNGQPENNYKTTPPVLDSDGSFFLYSKLTVDKSRWQQGNVFSCSVMHEALHNHYTQKSLSLSPGK

SEQ ID NO: 159 - protein, 449 aa, synthetic construct
EVQLVESGGGLVQPGRSLRLSCTASGSDINDYPITWVRQAPGQGLEWIGFINSGGSTWYASWVKGRFTISRDDSKSIAYLQMNSLKTEDTAVYYCARGYSTYYRDFNIWGQGTLVTVSSASTKGPSVFPLAPSSKSTSGGTAALGCLVKDYFPEPVTVSWNSGALTSGVHTFPAVLQSSGLYSLSSVVTVPSSSLGTQTYICNVNHKPSNTKVDKKVEPKSCDKTHTCPPCPAPELLGGPSVFLFPPKPKDTLMISRTPEVTCVVVDVSHEDPEVKFNWYVDGVEVHNAKTKPREEQYNSTYRVVSVLTVLHQDWLNGKEYKCKVSNKALPAPIEKTISKAKGQPREPQVYTLPPSREEMTKNQVSLTCLVKGFYPSDIAVEWESNGQPENNYKTTPPVLDSDGSFFLYSKLTVDKSRWQQGNVFSCSVMHEALHNHYTQKSLSLSPGK

SEQ ID NO: 160 - protein, 442 aa, synthetic construct
EVQLVQSGAEVKKPGESLRISCKGSGYSFSTYWISWVRQMPGKGLEWMGKIYPGDSYTNYSPSFQGQVTISADKSISTAYLQWSSLKASDTAMYYCARGYGIFDYWGQGTLVTVSSASTKGPSVFPLAPCSRSTSESTAALGCLVKDYFPEPVTVSWNSGALTSGVHTFPAVLQSSGLYSLSSVVTVPSSNFGTQTYTCNVDHKPSNTKVDKTVERKCCVECPPCPAPPVAGPSVFLFPPKPKDTLMISRTPEVTCVVVDVSHEDPEVQFNWYVDGVEVHNAKTKPREEQFNSTFRVVSVLTVVHQDWLNGKEYKCKVSNKGLPAPIEKTISKTKGQPREPQVYTLPPSREEMTKNQVSLTCLVKGFYPSDIAVEWESNGQPENNYKTTPPMLDSDGSFFLYSKLTVDKSRWQQGNVFSCSVMHEALHNHYTQKSLSLSPGK

SEQ ID NO: 161 - protein, 455 aa, synthetic construct
EVQLVESGGGLVQPGGSLKLSCAASGFTFNTYAMNWVRQASGKGLEWVGRIRSKYNNYATYYADSVKDRFTISRDDSKSTLYLQMNSLKTEDTAVYYCVRHGNFGNSYVSWFAYWGQGTLVTVSSASTKGPSVFPLAPSSKSTSGGTAALGCLVKDYFPEPVTVSWNSGALTSGVHTFPAVLQSSGLYSLSSVVTVPSSSLGTQTYICNVNHKPSNTKVDKKVEPKSCDKTHTCPPCPAPEAAGGPSVFLFPPKPKDTLMISRTPEVTCVVVDVSHEDPEVKFNWYVDGVEVHNAKTKPREEQYNSTYRVVSVLTVLHQDWLNGKEYKCKVSNKALPAPIEKTISKAKGQPREPQVYTLPPSREEMTKNQVSLTCLVKGFYPSDIAVEWESNGQPENNYKTTPPVLDSDGSFFLYSKLTVDKSRWQQGNVFSCSVMHEALHNHYTQKSLSLSPGK

SEQ ID NO: 162 - protein, 448 aa, synthetic construct
QVQLQQWGAGLLKPSETLSLTCAVYGGSFSGYYWSWIRQSPEKGLEWIGEINHGGYVTYNPSLESRVTISVDTSKNQFSLKLSSVTAADTAVYYCARDYGPGNYDWYFDLWGRGTLVTVSSASTKGPSVFPLAPCSRSTSESTAALGCLVKDYFPEPVTVSWNSGALTSGVHTFPAVLQSSGLYSLSSVVTVPSSSLGTKTYTCNVDHKPSNTKVDKRVESKYGPPCPPCPAPEFLGGPSVFLFPPKPKDTLMISRTPEVTCVVVDVSQEDPEVQFNWYVDGVEVHNAKTKPREEQFNSTYRVVSVLTVLHQDWLNGKEYKCKVSNKGLPSSIEKTISKAKGQPREPQVYTLPPSQEEMTKNQVSLTCLVKGFYPSDIAVEWESNGQPENNYKTTPPVLDSDGSFFLYSRLTVDKSRWQEGNVFSCSVMHEALHNHYTQKSLSLSLGK

SEQ ID NO: 163 - protein, 123 aa, synthetic construct
EVQLLESGGGLVQPGGSLRLSCAASGFTFRSFGMSWVRQAPGKGPEWVSSISGSGSDTLYADSVKGRFTISRDNSKNTLYLQMNSLRPEDTAVYYCTIGGSLSRSSQGTLVTVSSASHHHHHH

SEQ ID NO: 164 - protein, 450 aa, synthetic construct
QVQLVQSGAEVKKPGESLKVSCKASGYTFTSYYMHWVRQAPGQGLEWMGAIEPMYGSTSYAQKFQGRVTMTRDTSTSTVYMELSSLRSEDTAVYYCARGSAYYYDFADYWGQGTLVTVSSASTKGPSVFPLAPSSKSTSGGTAALGCLVKDYFPEPVTVSWNSGALTSGVHTFPAVLQSSGLYSLSSVVTVPSSSLGTQTYICNVNHKPSNTKVDKKVEPKSCDKTHTCPPCPAPEAAGGPSVFLFPPKPKDTLMISRTPEVTCVVVDVSHEDPEVKFNWYVDGVEVHNAKTKPREEQYNSTYRVVSVLTVLHQDWLNGKEYKCKVSNKALGAPIEKTISKAKGQPREPQVYTLPPSREEMTKNQVSLTCLVKGFYPSDIAVEWESNGQPENNYKTTPPVLDSDGSFFLYSKLTVDKSRWQQGNVFSCSVMHEALHNHYTQKSLSLSPGK

SEQ ID NO: 165 - protein, 450 aa, synthetic construct
QVQLVQSGAEVKKPGESLKVSCKASGYTFTSYYMHWVRQAPGQGLEWMGIINPSGGSTSYAQKFQGRVTMTRDTSTSTVYMELSSLRSEDTAVYYCARGSAYYYDFADYWGQGTLVTVSSASTKGPSVFPLAPSSKSTSGGTAALGCLVKDYFPEPVTVSWNSGALTSGVHTFPAVLQSSGLYSLSSVVTVPSSSLGTQTYICNVNHKPSNTKVDKKVEPKSCDKTHTCPPCPAPEAAGGPSVFLFPPKPKDTLMISRTPEVTCVVVDVSHEDPEVKFNWYVDGVEVHNAKTKPREEQYNSTYRVVSVLTVLHQDWLNGKEYKCKVSNKALGAPIEKTISKAKGQPREPQVYTLPPSREEMTKNQVSLTCLVKGFYPSDIAVEWESNGQPENNYKTTPPVLDSDGSFFLYSKLTVDKSRWQQGNVFSCSVMHEALHNHYTQKSLSLSPGK

SEQ ID NO: 166 - protein, 455 aa, synthetic construct
EVQLLESGGGLVQPGGSLRLSCAASGFTFSTYAMNWVRQAPGKGLEWVSRIRSKYNNYATYYADSVKDRFTISRDDSKSTLYLQMNSLRAEDTAVYYCVRHGNFGNSYVSWFAYWGQGTLVTVSSASTKGPSVFPLAPSSKSTSGGTAALGCLVKDYFPEPVTVSWNSGALTSGVHTFPAVLQSSGLYSLSSVVTVPSSSLGTQTYICNVNHKPSNTKVDKKVEPKSCDKTHTCPPCPAPEAAGGPSVFLFPPKPKDTLMISRTPEVTCVVVDVSHEDPEVKFNWYVDGVEVHNAKTKPREEQYNSTYRVVSVLTVLHQDWLNGKEYKCKVSNKALGAPIEKTISKAKGQPREPQVYTLPPSREEMTKNQVSLTCLVKGFYPSDIAVEWESNGQPENNYKTTPPVLDSDGSFFLYSKLTVDKSRWQQGNVFSCSVMHEALHNHYTQKSLSLSPGK

SEQ ID NO: 167 - protein, 214 aa, synthetic construct
DIQMTQSPSSLSASVGDRVTITCKASQGFNKYVAWYQQKPGKAPKLLIYYTSTLQPGVPSRFSGSGSGRDYTLTISSLQPEDFATYYCLQYGDLLYAFGQGTKVEIKRTVAAPSVFIFPPSDEQLKSGTASVVCLLNNFYPREAKVQWKVDNALQSGNSQESVTEQDSKDSTYSLSSTLTLSKADYEKHKVYACEVTHQGLSSPVTKSFNRGEC

SEQ ID NO: 168 - protein, 215 aa, synthetic construct
QAVVTQESALTTSPGETVTLTCRSSTGAVTTSNYANWVQEKPDHLFTGLIGGTNKRAPGVPARFSGSLIGDKAALTITGAQTEDEAIYFCALWYSNLWVFGGGTKLTVLGQPKAAPSVTLFPPSSEELQANKATLVCLISDFYPGAVTVAWKADSSPVKAGVETTTPSKQSNNKYAASSYLSLTPEQWKSHRSYSCQVTHEGSTVEKTVAPTECS

SEQ ID NO: 169 - protein, 214 aa, synthetic construct
DIQMTQSPSSLSASVGDRVTITCSASQDISNYLNWYQQKPGKAPKLLIYYTSNLHSGVPSRFSGSGSGTDFTLTISSLQPEDFATYYCQQYRKLPWTFGQGTKLEIKRTVAAPSVFIFPPSDEQLKSGTASVVCLLNNFYPREAKVQWKVDNALQSGNSQESVTEQDSKDSTYSLSSTLTLSKADYEKHKVYACEVTHQGLSSPVTKSFNRGEC

SEQ ID NO: 170 - protein, 212 aa, synthetic construct
DIVLTQSPAIMSASPGEKVTMTCSASSSVNYMYWYQQKSGTSPKRWIYDTSKLASGVPVRFSGSGSGTSYSLTISSMETEDAAEYYCQQWGRNPTFGGGTKLEIKRTVAAPSVFIFPPSDEQLKSGTASVVCLLNNFYPREAKVQWKVDNALQSGNSQESVTEQDSKDSTYSLSSTLTLSKADYEKHKVYACEVTHQGLSSPVTKSFNRGEC

SEQ ID NO: 171 - protein, 214 aa, synthetic construct
DIQMTQSPSSLSASVGDRVTITCKASQNVDTNVAWYQQKPGQAPKSLIYSASYRYSDVPSRFSGSASGTDFTLTISSVQSEDFATYYCQQYDSYPYTFGGGTKLEIKRTVAAPSVFIFPPSDEQLKSGTASVVCLLNNFYPREAKVQWKVDNALQSGNSQESVTEQDSKDSTYSLSSTLTLSKADYEKHKVYACEVTHQGLSSPVTKSFNRGEC

SEQ ID NO: 172 - protein, 217 aa, synthetic construct
DIQMTQSPSSLSASVGDRVTINCQASQSIDSNLAWFQQKPGQPPKLLIYRASNLASGVPDRFSGSGSGTDFTLTISSLEAEDVATYYCLGGVGAVSYRTSFGGGTKVEIKRTVAAPSVFIFPPSDEQLKSGTASVVCLLNNFYPREAKVQWKVDNALQSGNSQESVTEQDSKDSTYSLSSTLTLSKADYEKHKVYACEVTHQGLSSPVTKSFNRGEC

SEQ ID NO: 173 - protein, 214 aa, synthetic construct
SYELTQPPSVSVSPGQTASITCSGDNIGDQYAHWYQQKPGQSPVLVIYQDKNRPSGIPERFSGSNSGNTATLTISGTQAMDEADYYCATYTGFGSLAVFGGGTKLTVLGQPKAAPSVTLFPPSSEELQANKATLVCLISDFYPGAVTVAWKADSSPVKAGVETTTPSKQSNNKYAASSYLSLTPEQWKSHRSYSCQVTHEGSTVEKTVAPTECS

SEQ ID NO: 174 - protein, 215 aa, synthetic construct
QAVVTQEPSLTVSPGGTVTLTCRSSTGAVTTSNYANWVQQKPGQAPRGLIGGTNKRAPWTPARFSGSLLGDKAALTLLGAQPEDEAEYFCALWYSNLWVFGGGTKLTVLGQPKAAPSVTLFPPSSEELQANKATLVCLISDFYPGAVTVAWKADSSPVKAGVETTTPSKQSNNKYAASSYLSLTPEQWKSHRSYSCQVTHEGSTVEKTVAPTECS

SEQ ID NO: 175 - protein, 216 aa, synthetic construct
EIVLTQSPATLSLSPGERATLSCRASQSVSSYLAWYQQKPGQAPRLLIYDASNRATGIPARFSGSGSGTDFTLTISSLEPEDFAVYYCQQRSNWPPALTFGGGTKVEIKRTVAAPSVFIFPPSDEQLKSGTASVVCLLNNFYPREAKVQWKVDNALQSGNSQESVTEQDSKDSTYSLSSTLTLSKADYEKHKVYACEVTHQGLSSPVTKSFNRGEC

SEQ ID NO: 176 - protein, 212 aa, synthetic construct
SYVLTQPSSVSVAPGQTATISCGGHNIGSKNVHWYQQRPGQSPVLVIYQDNKRPSGIPERFSGSNSGNTATLTISGTQAMDEADYYCQVWDNYSVLFGGGTKLTVLGQPKAAPSVTLFPPSSEELQANKATLVCLISDFYPGAVTVAWKADSSPVKAGVETTTPSKQSNNKYAASSYLSLTPEQWKSHRSYSCQVTHEGSTVEKTVAPTECS

SEQ ID NO: 177 - protein, 224 aa, synthetic construct
EVQLVQSGAEVKKPGASVKVSCKASGYTFTSYWIGWVRQAPGQGLEWIGDIYPGGGYTNYNEKFKGRVTITRDTSTSTAYLELSSLRSEDTAVYYCARLAGSSYRGAMDSWGQGTLVTVSSASTKGPSVFPLAPSSKSTSGGTAALGCLVKDYFPEPVTVSWNSGALTSGVHTFPAVLQSSGLYSLSSVVTVPSSSLGTQTYICNVNHKPSNTKVDKKVEPKSC

SEQ ID NO: 178 - protein, 442 aa, synthetic construct
DIQMTQSPSSLSASVGDRVTITCKASQGFNKYVAWYQQKPGKAPKLLIYYTSTLQPGVPSRFSGSGSGRDYTLTISSLQPEDFATYYCLQYGDLLYAFGQGTKVEIKRTVAAPSVFIFPPSDEQLKSGTASVVCLLNNFYPREAKVQWKVDNALQSGNSQESVTEQDSKDSTYSLSSTLTLSKADYEKHKVYACEVTHQGLSSPVTKSFNRGECEVQLVESGGGLVQPKGSLKLSCAASGFTFNTYAMNWVRQAPGKGLEWVARIRSKYNNYATYYADSVKDRFTISRDDSQSILYLQMNNLKTEDTAMYYCVRHGNFGNSYVSWFAYWGQGTLVTVSAASTKGPSVFPLAPSSKSTSGGTAALGCLVKDYFPEPVTVSWNSGALTSGVHTFPAVLQSSGLYSLSSVVTVPSSSLGTQTYICNVNHKPSNTKVDKKVEPKSC

SEQ ID NO: 179 - protein, 224 aa, synthetic construct
QVQLVESGGGLVKPGESLRLSCAASGFTFSDYYMYWVRQAPGKGLEWVAIISDGGYYTYYSDIIKGRFTISRDNAKNSLYLQMNSLKAEDTAVYYCARGFPLLRHGAMDYWGQGTLVTVSSASTKGPSVFPLAPSSKSTSGGTAALGCLVKDYFPEPVTVSWNSGALTSGVHTFPAVLQSSGLYSLSSVVTVPSSSLGTQTYICNVNHKPSNTKVDKKVEPKSC

SEQ ID NO: 180 - protein, 442 aa, synthetic construct
DIQMTQSPSSLSASVGDRVTITCKASQNVDTNVAWYQQKPGQAPKSLIYSASYRYSDVPSRFSGSASGTDFTLTISSVQSEDFATYYCQQYDSYPYTFGGGTKLEIKRTVAAPSVFIFPPSDEQLKSGTASVVCLLNNFYPREAKVQWKVDNALQSGNSQESVTEQDSKDSTYSLSSTLTLSKADYEKHKVYACEVTHQGLSSPVTKSFNRGECEVQLVESGGGLVQPGGSLKLSCAASGFTFNTYAMNWVRQASGKGLEWVGRIRSKYNNYATYYADSVKDRFTISRDDSKSTLYLQMNSLKTEDTAVYYCVRHGNFGNSYVSWFAYWGQGTLVTVSSASTKGPSVFPLAPSSKSTSGGTAALGCLVKDYFPEPVTVSWNSGALTSGVHTFPAVLQSSGLYSLSSVVTVPSSSLGTQTYICNVNHKPSNTKVDKKVEPKSC

SEQ ID NO: 181 - protein, 224 aa, synthetic construct
QVQLVQSGAEVKKPGSSVKVSCKASGGTFSNYWMHWVRQAPGQGLEWMGATYRGHSDTYYNQKFKGRVTITADKSTSTAYMELSSLRSEDTAVYYCARGAIYDGYDVLDNWGQGTLVTVSSASTKGPSVFPLAPSSKSTSGGTAALGCLVKDYFPEPVTVSWNSGALTSGVHTFPAVLQSSGLYSLSSVVTVPSSSLGTQTYICNVNHKPSNTKVDKKVEPKSC

SEQ ID NO: 182 - protein, 442 aa, synthetic construct
DIQMTQSPSSLSASVGDRVTITCSASQDISNYLNWYQQKPGKAPKLLIYYTSNLHSGVPSRFSGSGSGTDFTLTISSLQPEDFATYYCQQYRKLPWTFGQGTKLEIKRTVAAPSVFIFPPSDEQLKSGTASVVCLLNNFYPREAKVQWKVDNALQSGNSQESVTEQDSKDSTYSLSSTLTLSKADYEKHKVYACEVTHQGLSSPVTKSFNRGECEVQLVESGGGLVQPGGSLKLSCAASGFTFNTYAMNWVRQASGKGLEWVGRIRSKYNNYATYYADSVKDRFTISRDDSKSTLYLQMNSLKTEDTAVYYCVRHGNFGNSYVSWFAYWGQGTLVTVSSASTKGPSVFPLAPSSKSTSGGTAALGCLVKDYFPEPVTVSWNSGALTSGVHTFPAVLQSSGLYSLSSVVTVPSSSLGTQTYICNVNHKPSNTKVDKKVEPKSC

SEQ ID NO: 183 - protein, 222 aa, synthetic construct
EVQLVESGGGLVQPGRSLRLSCTASGSDINDYPITWVRQAPGQGLEWIGFINSGGSTWYASWVKGRFTISRDDSKSIAYLQMNSLKTEDTAVYYCARGYSTYYRDFNIWGQGTLVTVSSASTKGPSVFPLAPSSKSTSGGTAALGCLVKDYFPEPVTVSWNSGALTSGVHTFPAVLQSSGLYSLSSVVTVPSSSLGTQTYICNVNHKPSNTKVDKKVEPKSC

SEQ ID NO: 184 - protein, 445 aa, synthetic construct
DIQMTQSPSSLSASVGDRVTINCQASQSIDSNLAWFQQKPGQPPKLLIYRASNLASGVPDRFSGSGSGTDFTLTISSLEAEDVATYYCLGGVGAVSYRTSFGGGTKVEIKRTVAAPSVFIFPPSDEQLKSGTASVVCLLNNFYPREAKVQWKVDNALQSGNSQESVTEQDSKDSTYSLSSTLTLSKADYEKHKVYACEVTHQGLSSPVTKSFNRGECEVQLVESGGGLVQPGGSLKLSCAASGFTFNTYAMNWVRQASGKGLEWVGRIRSKYNNYATYYADSVKDRFTISRDDSKSTLYLQMNSLKTEDTAVYYCVRHGNFGNSYVSWFAYWGQGTLVTVSSASTKGPSVFPLAPSSKSTSGGTAALGCLVKDYFPEPVTVSWNSGALTSGVHTFPAVLQSSGLYSLSSVVTVPSSSLGTQTYICNVNHKPSNTKVDKKVEPKSC

SEQ ID NO: 185 - protein, 219 aa, synthetic construct
EVQLQQSGAELMKPGASVKISCKASGYTFSDYWIEWVKQRPGHGLEWIGEILPGSGSTNYHERFKGKATFTADTSSSTAYMQLNSLTSEDSGVYYCLHGNYDFDGWGQGTTLTVSSASTKGPSVFPLAPSSKSTSGGTAALGCLVKDYFPEPVTVSWNSGALTSGVHTFPAVLQSSGLYSLSSVVTVPSSSLGTQTYICNVNHKPSNTKVDKKVEPKSC

SEQ ID NO: 186 - protein, 440 aa, synthetic construct
DIVLTQSPAIMSASPGEKVTMTCSASSSVNYMYWYQQKSGTSPKRWIYDTSKLASGVPVRFSGSGSGTSYSLTISSMETEDAAEYYCQQWGRNPTFGGGTKLEIKRTVAAPSVFIFPPSDEQLKSGTASVVCLLNNFYPREAKVQWKVDNALQSGNSQESVTEQDSKDSTYSLSSTLTLSKADYEKHKVYACEVTHQGLSSPVTKSFNRGECEVQLVESGGGLVQPGGSLKLSCAASGFTFNTYAMNWVRQASGKGLEWVGRIRSKYNNYATYYADSVKDRFTISRDDSKSTLYLQMNSLKTEDTAVYYCVRHGNFGNSYVSWFAYWGQGTLVTVSSASTKGPSVFPLAPSSKSTSGGTAALGCLVKDYFPEPVTVSWNSGALTSGVHTFPAVLQSSGLYSLSSVVTVPSSSLGTQTYICNVNHKPSNTKVDKKVEPKSC

SEQ ID NO: 187 - protein, 567 aa, synthetic construct
DIQMTQSPSSLSASVGDRVTITCKASQGFNKYVAWYQQKPGKAPKLLIYYTSTLQPGVPSRFSGSGSGRDYTLTISSLQPEDFATYYCLQYGDLLYAFGQGTKVEIKRTVAAPSVFIFPPSDEQLKSGTASVVCLLNNFYPREAKVQWKVDNALQSGNSQESVTEQDSKDSTYSLSSTLTLSKADYEKHKVYACEVTHQGLSSPVTKSFNRGECEVQLVESGGGLVQPGGSLKLSCAASGFTFNTYAMNWVRQASGKGLEWVGRIRSKYNNYATYYADSVKDRFTISRDDSKSTLYLQMNSLKTEDTAVYYCVRHGNFGNSYVSWFAYWGQGTLVTVSSASTKGPSVFPLAPSSKSTSGGTAALGCLVKDYFPEPVTVSWNSGALTSGVHTFPAVLQSSGLYSLSSVVTVPSSSLGTQTYICNVNHKPSNTKVDKKVEPKSCGGGGSGGGGSEVQLLESGGGLVQPGGSLRLSCAASGFTFRSFGMSWVRQAPGKGPEWVSSISGSGSDTLYADSVKGRFTISRDNSKNTLYLQMNSLRPEDTAVYYCTIGGSLSRSSQGTLVTVSS

SEQ ID NO: 188 - protein, 437 aa, synthetic construct
DIQMTQSPSSLSASVGDRVTITCKASQGFNKYVAWYQQKPGKAPKLLIYYTSTLQPGVPSRFSGSGSGRDYTLTISSLQPEDFATYYCLQYGDLLYAFGQGTKVEIKRTVAAPSVFIFPPSDEQLKSGTASVVCLLNNFYPREAKVQWKVDNALQSGNSQESVTEQDSKDSTYSLSSTLTLSKADYEKHKVYACEVTHQGLSSPVTKSFNRGECQVQLVQSGAEVKKPGESLKVSCKASGYTFTSYYMHWVRQAPGQGLEWMGAIEPMYGSTSYAQKFQGRVTMTRDTSTSTVYMELSSLRSEDTAVYYCARGSAYYYDFADYWGQGTLVTVSSASTKGPSVFPLAPSSKSTSGGTAALGCLVKDYFPEPVTVSWNSGALTSGVHTFPAVLQSSGLYSLSSVVTVPSSSLGTQTYICNVNHKPSNTKVDKKVEPKSC

SEQ ID NO: 189 - protein, 437 aa, synthetic construct
DIQMTQSPSSLSASVGDRVTITCKASQGFNKYVAWYQQKPGKAPKLLIYYTSTLQPGVPSRFSGSGSGRDYTLTISSLQPEDFATYYCLQYGDLLYAFGQGTKVEIKRTVAAPSVFIFPPSDEQLKSGTASVVCLLNNFYPREAKVQWKVDNALQSGNSQESVTEQDSKDSTYSLSSTLTLSKADYEKHKVYACEVTHQGLSSPVTKSFNRGECQVQLVQSGAEVKKPGESLKVSCKASGYTFTSYYMHWVRQAPGQGLEWMGIINPSGGSTSYAQKFQGRVTMTRDTSTSTVYMELSSLRSEDTAVYYCARGSAYYYDFADYWGQGTLVTVSSASTKGPSVFPLAPSSKSTSGGTAALGCLVKDYFPEPVTVSWNSGALTSGVHTFPAVLQSSGLYSLSSVVTVPSSSLGTQTYICNVNHKPSNTKVDKKVEPKSC

SEQ ID NO: 190 - protein, 437 aa, synthetic construct
DIQMTQSPSSLSASVGDRVTITCSASQDISNYLNWYQQKPGKAPKLLIYYTSNLHSGVPSRFSGSGSGTDFTLTISSLQPEDFATYYCQQYRKLPWTFGQGTKLEIKRTVAAPSVFIFPPSDEQLKSGTASVVCLLNNFYPREAKVQWKVDNALQSGNSQESVTEQDSKDSTYSLSSTLTLSKADYEKHKVYACEVTHQGLSSPVTKSFNRGECQVQLVQSGAEVKKPGESLKVSCKASGYTFTSYYMHWVRQAPGQGLEWMGAIEPMYGSTSYAQKFQGRVTMTRDTSTSTVYMELSSLRSEDTAVYYCARGSAYYYDFADYWGQGTLVTVSSASTKGPSVFPLAPSSKSTSGGTAALGCLVKDYFPEPVTVSWNSGALTSGVHTFPAVLQSSGLYSLSSVVTVPSSSLGTQTYICNVNHKPSNTKVDKKVEPKSC

SEQ ID NO: 191 - protein, 437 aa, synthetic construct
DIQMTQSPSSLSASVGDRVTITCSASQDISNYLNWYQQKPGKAPKLLIYYTSNLHSGVPSRFSGSGSGTDFTLTISSLQPEDFATYYCQQYRKLPWTFGQGTKLEIKRTVAAPSVFIFPPSDEQLKSGTASVVCLLNNFYPREAKVQWKVDNALQSGNSQESVTEQDSKDSTYSLSSTLTLSKADYEKHKVYACEVTHQGLSSPVTKSFNRGECQVQLVQSGAEVKKPGESLKVSCKASGYTFTSYYMHWVRQAPGQGLEWMGIINPSGGSTSYAQKFQGRVTMTRDTSTSTVYMELSSLRSEDTAVYYCARGSAYYYDFADYWGQGTLVTVSSASTKGPSVFPLAPSSKSTSGGTAALGCLVKDYFPEPVTVSWNSGALTSGVHTFPAVLQSSGLYSLSSVVTVPSSSLGTQTYICNVNHKPSNTKVDKKVEPKSC

SEQ ID NO: 192 - protein, 215 aa, synthetic construct
EIVLTQSPATLSLSPGERATLSCRASQSVSSYLAWYQQKPGQAPRLLIYDASNRATGIPARFSGSGSGTDFTLTISSLEPEDFAVYYCQQRSNWPPALTFGGGTKVTVLGQPKAAPSVTLFPPSSEELQANKATLVCLISDFYPGAVTVAWKADSSPVKAGVETTTPSKQSNNKYAASSYLSLTPEQWKSHRSYSCQVTHEGSTVEKTVAPTECS

SEQ ID NO: 193 - protein, 436 aa, synthetic construct
DIVLTQSPAIMSASPGEKVTMTCSASSSVNYMYWYQQKSGTSPKRWIYDTSKLASGVPVRFSGSGSGTSYSLTISSMETEDAAEYYCQQWGRNPTFGGGTKLEIKRTVAAPSVFIFPPSDEQLKSGTASVVCLLNNFYPREAKVQWKVDNALQSGNSQESVTEQDSKDSTYSLSSTLTLSKADYEKHKVYACEVTHQGLSSPVTKSFNRGECQVQLQQWGAGLLKPSETLSLTCAVYGGSFSGYYWSWIRQSPEKGLEWIGEINHGGYVTYNPSLESRVTISVDTSKNQFSLKLSSVTAADTAVYYCARDYGPGNYDWYFDLWGRGTLVTVSSASTKGPSVFPLAPSSKSTSGGTAALGCLVKDYFPEPVTVSWNSGALTSGVHTFPAVLQSSGLYSLSSVVTVPSSSLGTQTYICNVNHKPSNTKVDKKVEPKSC

SEQ ID NO: 194 - protein, 431 aa, synthetic construct
DIVLTQSPAIMSASPGEKVTMTCSASSSVNYMYWYQQKSGTSPKRWIYDTSKLASGVPVRFSGSGSGTSYSLTISSMETEDAAEYYCQQWGRNPTFGGGTKLEIKRTVAAPSVFIFPPSDEQLKSGTASVVCLLNNFYPREAKVQWKVDNALQSGNSQESVTEQDSKDSTYSLSSTLTLSKADYEKHKVYACEVTHQGLSSPVTKSFNRGECEVQLVQSGAEVKKPGESLRISCKGSGYSFSTYWISWVRQMPGKGLEWMGKIYPGDSYTNYSPSFQGQVTISADKSISTAYLQWSSLKASDTAMYYCARGYGIFDYWGQGTLVTVSSASTKGPSVFPLAPSSKSTSGGTAALGCLVKDYFPEPVTVSWNSGALTSGVHTFPAVLQSSGLYSLSSVVTVPSSSLGTQTYICNVNHKPSNTKVDKKVEPKSC

SEQ ID NO: 195 - protein, 438 aa, synthetic construct
DIQMTQSPSSLSASVGDRVTITCKASQGFNKYVAWYQQKPGKAPKLLIYYTSTLQPGVPSRFSGSGSGRDYTLTISSLQPEDFATYYCLQYGDLLYAFGQGTKVEIKRTVAAPSVFIFPPSDEQLKSGTASVVCLLNNFYPREAKVQWKVDNALQSGNSQESVTEQDSKDSTYSLSSTLTLSKADYEKHKVYACEVTHQGLSSPVTKSFNRGECQVQLQQWGAGLLKPSETLSLTCAVYGGSFSGYYWSWIRQSPEKGLEWIGEINHGGYVTYNPSLESRVTISVDTSKNQFSLKLSSVTAADTAVYYCARDYGPGNYDWYFDLWGRGTLVTVSSASTKGPSVFPLAPSSKSTSGGTAALGCLVKDYFPEPVTVSWNSGALTSGVHTFPAVLQSSGLYSLSSVVTVPSSSLGTQTYICNVNHKPSNTKVDKKVEPKSC

SEQ ID NO: 196 - protein, 433 aa, synthetic construct
DIQMTQSPSSLSASVGDRVTITCKASQGFNKYVAWYQQKPGKAPKLLIYYTSTLQPGVPSRFSGSGSGRDYTLTISSLQPEDFATYYCLQYGDLLYAFGQGTKVEIKRTVAAPSVFIFPPSDEQLKSGTASVVCLLNNFYPREAKVQWKVDNALQSGNSQESVTEQDSKDSTYSLSSTLTLSKADYEKHKVYACEVTHQGLSSPVTKSFNRGECEVQLVQSGAEVKKPGESLRISCKGSGYSFSTYWISWVRQMPGKGLEWMGKIYPGDSYTNYSPSFQGQVTISADKSISTAYLQWSSLKASDTAMYYCARGYGIFDYWGQGTLVTVSSASTKGPSVFPLAPSSKSTSGGTAALGCLVKDYFPEPVTVSWNSGALTSGVHTFPAVLQSSGLYSLSSVVTVPSSSLGTQTYICNVNHKPSNTKVDKKVEPKSC